European Patent Application EP 4 620 966 A1, published September 24, 2025. Title: Peptide having activities of skin condition improvement and uses thereof. Applicant: CAREGEN CO., LTD. The sequence listing filed with the application follows.

SEQUENCE LISTING (13 sequences)

SEQ ID NO: 1 - protein, 5 aa, synthetic construct
DGWNY

SEQ ID NO: 2 - DNA, 20 bp, synthetic construct
  source 1..20: mol_type = other DNA
caccctcaagagcctgagtc

SEQ ID NO: 3 - DNA, 20 bp, synthetic construct
  source 1..20: mol_type = other DNA
agacggctgagtagggaaca

SEQ ID NO: 4 - DNA, 20 bp, synthetic construct
  source 1..20: mol_type = other DNA
ccaggaaccgagtacaccat

SEQ ID NO: 5 - DNA, 20 bp, synthetic construct
  source 1..20: mol_type = other DNA
atacccaggttgggtgatga

SEQ ID NO: 6 - DNA, 20 bp, synthetic construct
  source 1..20: mol_type = other DNA
gcaagacctggctttggact

SEQ ID NO: 7 - DNA, 21 bp, synthetic construct
  source 1..21: mol_type = other DNA
gggagtttctggttagggctg

SEQ ID NO: 8 - DNA, 20 bp, synthetic construct
  source 1..20: mol_type = other DNA
ggagccaaaagggtcatcat

SEQ ID NO: 9 - DNA, 20 bp, synthetic construct
  source 1..20: mol_type = other DNA
gtgatggcatggactgtggt

SEQ ID NO: 10 - DNA, 20 bp, synthetic construct
  source 1..20: mol_type = other DNA
tcagtggctggaacagtgag

SEQ ID NO: 11 - DNA, 20 bp, synthetic construct
  source 1..20: mol_type = other DNA
tctggcatgtcccactatca

SEQ ID NO: 12 - DNA, 20 bp, synthetic construct
  source 1..20: mol_type = other DNA
ccttcttgggtgctggaata

SEQ ID NO: 13 - DNA, 20 bp, synthetic construct
  source 1..20: mol_type = other DNA
acacgataagggaggctgtg